European Patent Application EP 4 374 874 A1, published May 29, 2024. Title: PHARMACEUTICAL COMPOSITION CONTAINING ANTI-TROP2 ANTIBODY DRUG CONJUGATE AND ITS APPLICATION. Applicant: JIANGSU HENGRUI PHARMACEUTICALS CO., LTD. Application WO PCT/CN2022/107134, filed July 21, 2022. The sequence listing filed with the application follows.

SEQUENCE LISTING (6 sequences)

SEQ ID NO: 1 - protein, 451 aa, synthetic construct
  CHAIN 1..451: note = HC
EVQLVQSGSELKKPGASVKVSCKASGYTFTNYGMNWVKQAPGQGLKWMGWINTYTGEPTYTQDFKGRFAFSLDTSVSTAYLQISSLKAEDTAVYYCARGGFGSSYWYFDVWGQGTLVTVSSASTKGPSVFPLAPSSKSTSGGTAALGCLVKDYFPEPVTVSWNSGALTSGVHTFPAVLQSSGLYSLSSVVTVPSSSLGTQTYICNVNHKPSNTKVDKKVEPKSCDKTHTCPPCPAPELLGGPSVFLFPPKPKDTLMISRTPEVTCVVVDVSHEDPEVKFNWYVDGVEVHNAKTKPREEQYNSTYRVVSVLTVLHQDWLNGKEYKCKVSNKALPAPIEKTISKAKGQPREPQVYTLPPSRDELTKNQVSLTCLVKGFYPSDIAVEWESNGQPENNYKTTPPVLDSDGSFFLYSKLTVDKSRWQQGNVFSCSVMHEALHNHYTQKSLSLSPGK

SEQ ID NO: 2 - protein, 214 aa, synthetic construct
  CHAIN 1..214: note = LC
DIQLTQSPSSLSASVGDRVSITCKASQDVSIAVAWYQQKPGKAPKLLIYSASYRYTGVPDRFSGSGSGTDFTLTISSLQPEDFAVYYCQQHYITPLTFGAGTKVEIKRTVAAPSVFIFPPSDEQLKSGTASVVCLLNNFYPREAKVQWKVDNALQSGNSQESVTEQDSKDSTYSLSSTLTLSKADYEKHKVYACEVTHQGLSSPVTKSFNRGEC

SEQ ID NO: 3 - protein, 451 aa, synthetic construct
  CHAIN 1..451: note = HC
QVQLQQSGSELKKPGASVKVSCKASGYTFTNYGMNWVKQAPGQGLKWMGWINTYTGEPTYTDDFKGRFAFSLDTSVSTAYLQISSLKADDTAVYFCARGGFGSSYWYFDVWGQGSLVTVSSASTKGPSVFPLAPSSKSTSGGTAALGCLVKDYFPEPVTVSWNSGALTSGVHTFPAVLQSSGLYSLSSVVTVPSSSLGTQTYICNVNHKPSNTKVDKKVEPKSCDKTHTCPPCPAPELLGGPSVFLFPPKPKDTLMISRTPEVTCVVVDVSHEDPEVKFNWYVDGVEVHNAKTKPREEQYNSTYRVVSVLTVLHQDWLNGKEYKCKVSNKALPAPIEKTISKAKGQPREPQVYTLPPSRDELTKNQVSLTCLVKGFYPSDIAVEWESNGQPENNYKTTPPVLDSDGSFFLYSKLTVDKSRWQQGNVFSCSVMHEALHNHYTQKSLSLSPGK

SEQ ID NO: 4 - protein, 214 aa, synthetic construct; identical to SEQ ID NO: 2
  CHAIN 1..214: note = LC

SEQ ID NO: 5 - protein, 451 aa, synthetic construct
  CHAIN 1..451: note = HC
QVQLVQSGAEVKKPGASVKVSCKASGYTFTTAGMQWVRQAPGQGLEWMGWINTHSGVPKYAEDFKGRVTISADTSTSTAYLQLSSLKSEDTAVYYCARSGFGSSYWYFDVWGQGTLVTVSSASTKGPSVFPLAPSSKSTSGGTAALGCLVKDYFPEPVTVSWNSGALTSGVHTFPAVLQSSGLYSLSSVVTVPSSSLGTQTYICNVNHKPSNTKVDKKVEPKSCDKTHTCPPCPAPELLGGPSVFLFPPKPKDTLMISRTPEVTCVVVDVSHEDPEVKFNWYVDGVEVHNAKTKPREEQYNSTYRVVSVLTVLHQDWLNGKEYKCKVSNKALPAPIEKTISKAKGQPREPQVYTLPPSRDELTKNQVSLTCLVKGFYPSDIAVEWESNGQPENNYKTTPPVLDSDGSFFLYSKLTVDKSRWQQGNVFSCSVMHEALHNHYTQKSLSLSPGK

SEQ ID NO: 6 - protein, 214 aa, synthetic construct
  CHAIN 1..214: note = LC
DIQMTQSPSSLSASVGDRVTITCKASQDVSTAVAWYQQKPGKAPKLLIYSASYRYTGVPSRFSGSGSGTDFTLTISSLQPEDFAVYYCQQHYITPLTFGQGTKLEIKRTVAAPSVFIFPPSDEQLKSGTASVVCLLNNFYPREAKVQWKVDNALQSGNSQESVTEQDSKDSTYSLSSTLTLSKADYEKHKVYACEVTHQGLSSPVTKSFNRGEC